European Patent Application EP 4 201 407 A1, published June 28, 2023. Title: MITOCHONDRIAL-TARGETED ANTIOXIDANT AS A THERAPEUTIC AGENT FOR PATHOLOGICAL INFLAMMATION CAUSED BY MABC-R INFECTION. Applicant: MitoImmune Therapeutics Inc. The sequence listing filed with the application follows.

SEQUENCE LISTING (30 sequences)

SEQ ID NO: 1 - protein, 20 aa, Artificial Sequence
  forward primer for Tnf
  BINDING (1)..(20): forward primer for Tnf
ACGGCATGGATCTCAAAGAC

SEQ ID NO: 2 - protein, 20 aa, Artificial Sequence
  reverse primer for Tnf
  BINDING (1)..(20): reverse primer for Tnf
AGATAGCAAATCGGCTGACG

SEQ ID NO: 3 - protein, 22 aa, Artificial Sequence
  forward primer for Il6
  BINDING (1)..(22): forward primer for Il6
TACCACTTCACAAGTCGGAGGC

SEQ ID NO: 4 - protein, 23 aa, Artificial Sequence
  reverse primer for Il6
  BINDING (1)..(23): reverse primer for Il6
CTGCAAGTGCATCATCGTTGTTC

SEQ ID NO: 5 - protein, 22 aa, Artificial Sequence
  forward primer for Il12p40
  BINDING (1)..(22): forward primer for Il12p40
TTGAACTGGCGTTGGAAGCACG

SEQ ID NO: 6 - protein, 23 aa, Artificial Sequence
  reverse primer for Il12p40
  BINDING (1)..(23): reverse primer for Il12p40
CCACCTGTGAGTTCTTCAAAGGC

SEQ ID NO: 7 - protein, 19 aa, Artificial Sequence
  forward primer for Il1b
  BINDING (1)..(19): forward primer for Il1b
TACGGACCCCAAAAGATGA

SEQ ID NO: 8 - protein, 20 aa, Artificial Sequence
  reverse primer for Il1b
  BINDING (1)..(20): reverse primer for Il1b
TGCTGCTGCGAGATTTGAAG

SEQ ID NO: 9 - protein, 20 aa, Artificial Sequence
  forward primer for Ifng
  BINDING (1)..(20): forward primer for Ifng
CGGCACAGTCATTGAAAGCC

SEQ ID NO: 10 - protein, 20 aa, Artificial Sequence
  reverse primer for Ifng
  BINDING (1)..(20): reverse primer for Ifng
TGCATCCTTTTTCGCCTTGC

SEQ ID NO: 11 - protein, 20 aa, Artificial Sequence
  forward primer for Ccl2
  BINDING (1)..(20): forward primer for Ccl2
TGACCCCAAGAAGGAATGGG

SEQ ID NO: 12 - protein, 20 aa, Artificial Sequence
  reverse primer for Ccl2
  BINDING (1)..(20): reverse primer for Ccl2
ACCTTAGGGCAGATGCAGTT

SEQ ID NO: 13 - protein, 20 aa, Artificial Sequence
  forward primer for Cxcl2
  BINDING (1)..(20): forward primer for Cxcl2
CCCTGCCAAGGGTTGACTTC

SEQ ID NO: 14 - protein, 20 aa, Artificial Sequence
  reverse primer for Cxcl2
  BINDING (1)..(20): reverse primer for Cxcl2
GCAAACTTTTTGACCGCCCT

SEQ ID NO: 15 - protein, 22 aa, Artificial Sequence
  forward primer for Cxcl5
  BINDING (1)..(22): forward primer for Cxcl5
CCGCTGGCATTTCTGTTGCTGT

SEQ ID NO: 16 - protein, 23 aa, Artificial Sequence
  reverse primer for Cxcl5
  BINDING (1)..(23): reverse primer for Cxcl5
CAGGGATCACCTCCAAATTAGCG

SEQ ID NO: 17 - protein, 22 aa, Artificial Sequence
  forward primer for Sirt3
  BINDING (1)..(22): forward primer for Sirt3
GCTACATGCACGGTCTGTCGAA

SEQ ID NO: 18 - protein, 22 aa, Artificial Sequence
  reverse primer for Sirt3
  BINDING (1)..(22): reverse primer for Sirt3
CAATGTCGGGTTTCACAACGCC

SEQ ID NO: 19 - protein, 22 aa, Artificial Sequence
  forward primer for Ndufab1
  BINDING (1)..(22): forward primer for Ndufab1
GGACCGAGTTCTGTATGTCTTG

SEQ ID NO: 20 - protein, 22 aa, Artificial Sequence
  reverse primer for Ndufab1
  BINDING (1)..(22): reverse primer for Ndufab1
AAACCCAAATTCGTCTTCCATG

SEQ ID NO: 21 - protein, 19 aa, Artificial Sequence
  forward primer for Sdhb
  BINDING (1)..(19): forward primer for Sdhb
ACCCCTTCTCTGTCTACCG

SEQ ID NO: 22 - protein, 21 aa, Artificial Sequence
  reverse primer for Sdhb
  BINDING (1)..(21): reverse primer for Sdhb
AATGCTCGCTTCTCCTTGTAG

SEQ ID NO: 23 - protein, 19 aa, Artificial Sequence
  forward primer for Uqcrc1
  BINDING (1)..(19): forward primer for Uqcrc1
ATCAAGGCACTGTCCAAGG

SEQ ID NO: 24 - protein, 20 aa, Artificial Sequence
  reverse primer for Uqcrc1
  BINDING (1)..(20): reverse primer for Uqcrc1
TCATTTTCCTGCATCTCCCG

SEQ ID NO: 25 - protein, 20 aa, Artificial Sequence
  forward primer for Cox5b
  BINDING (1)..(20): forward primer for Cox5b
ACCCTAATCTAGTCCCGTCC

SEQ ID NO: 26 - protein, 20 aa, Artificial Sequence
  reverse primer for Cox5b
  BINDING (1)..(20): reverse primer for Cox5b
CAGCCAAAACCAGATGACAG

SEQ ID NO: 27 - protein, 20 aa, Artificial Sequence
  forward primer for Atp5a1
  BINDING (1)..(20): forward primer for Atp5a1
CATTGGTGATGGTATTGCGC

SEQ ID NO: 28 - protein, 19 aa, Artificial Sequence
  reverse primer for Atp5a1
  BINDING (1)..(19): reverse primer for Atp5a1
TCCCAAACACGACAACTCC

SEQ ID NO: 29 - protein, 21 aa, Artificial Sequence
  forward primer for Gapdh
  BINDING (1)..(21): forward primer for Gapdh
AAGATGGTGATGGGCTTCCCG

SEQ ID NO: 30 - protein, 22 aa, Artificial Sequence
  reverse primer for Gapdh
  BINDING (1)..(22): reverse primer for Gapdh
TGGCAAAGTGGAGATTGTTGCC